European Patent Specification EP 3 497 213 B1, published October 18, 2023. Title: CELLULOSE SYNTHASE INHIBITORS AND MUTANT PLANTS. Applicant: VIB VZW UNIVERSITEIT GENT. The sequence listing filed with the application follows.

SEQUENCE LISTING (16 sequences)

SEQ ID NO: 1 - DNA, 55 bp, Artificial Sequence
  Primer
ggggacaagtttgtacaaaaaagcaggcttcatggaatccgaaggagaaaccgcg

SEQ ID NO: 2 - DNA, 52 bp, Artificial Sequence
  Primer
ggggaccactttgtacaagaaagctgggtgtcgcttctcaacagttgattcc

SEQ ID NO: 3 - protein, 249 aa, Arabidopsis thaliana
LTPYRVVIILRLIILCFFLQYRTTHPVKNAYPLWLTSVICEIWFAFSWLLITSIPLIAYCILPAFCLITDRFIIPEISNYASIWFILLFISIAVTGILELRWSGVSIEDWWRNEQFWVIGGTSAHLFAVFQGLLKVLAGIDTNFTVTSKATDEDGDFAELYIFKWTALLIPPTTVLLVNLIGIVAGVSYAVNSGYQSWGPLFGKLFFALWVIAHLYPFLKGLLGRQNRTPTIVIVWSVLLASIFSLLWV

SEQ ID NO: 4 - protein, 249 aa, Glycine max
LTPYRVVIILRLIILGFFLQYRVTHPVKDAYPLWLTSVICEIWFALSWLLFTSIPLIAYCTLPAFCLLTNKFIIPEISNFASMWFILLFVSIFTTSILELRWSGVSIEDWWRNEQFWVIGGTSAHLFAVFQGLLKVLAGIDTNFTVTSKASDEDGDFAELYVFKWTSLLIPPTTVLIVNLVGIVAGVSYAINSGYQSWGPLFGKLFFAIWVIAHLYPFLKGLLGRQNRTPTIVIVWSVLLASIFSLLWV

SEQ ID NO: 5 - protein, 249 aa, Fragaria vesca
LTPYRVVIILRLIILCFFLQYRATHPVKDAYPLWLISVICEIWFAFSWLLLTSIPLIAYCMLPAFCLLTNKFIIPEISNFASMWFILLFVSIAATGILELRWSGVGIDDWWRNEQFWVIGGTSAHLFAVFQGLLKVLAGIDTNFTVTSKASDEDGDFAELYVFKWTSLLIPPTTVLIVNLVGIVAGVSYAINSGYQSWGPLFGKLFFAMWVVAHLYPFLKGLLGRQNRTPTIVIVWSILLASIFSLLWV

SEQ ID NO: 6 - protein, 249 aa, Vitis vinifera
LTPYRVVIILRLIILGFFLQYRTTHPVKDAYPLWLTSVICEIWFALSWLLLTSIPLIAYCVLPAICLLTGKFIIPEISNFASMWFILLFVSIFATGILELRWSGVSIEDWWRNEQFWVIGGTSAHLFAVFQGLLKVLAGIDTNFTVTSKASDDDGDFAELYVFKWTSLLIPPTTVLVVNLVGIVAGVSYAINSGYQSWGPLFGKLFFAIWVIVHLYPFLKGLLGRQNRTPTIVIVWSILLASIFSLLWV

SEQ ID NO: 7 - protein, 249 aa, Solanum lycopersicum
LTPYRVVIILRLIILGFFMQYRLTHPVNDAYPLWLVSVICEVWFALSWLLLTSLPLLAYCTLPAICLLTGKFIIPEISNYAGMWFILLFLSIFATGILELRWSGVSIEDWWRNEQFWVIGGTSAHLFAVFQGLLKVLAGIDTNFTVTSKANDEDGDFAELYVFKWTTLLIPPTAILIVNLVGIVAGVSYAINSGYQSWGPLFGKLFFAIWVIVHLYPFLKGLLGRQNRTPTIVIVWAVLLASIFSLLWV

SEQ ID NO: 8 - protein, 249 aa, Zea mays
LNLYRVVIILRLIILCFFFQYRVSHPVRDAYGLWLVSVICEVWFALSWLLITSIPLIAYCVLPAICLLTNKFIIPEISNYAGMFFILLFASIFATGILELRWSGVGIEDWWRNEQFWVIGGTSAHLFAVFQGLLKVLAGIDTNFTVTSKASDEDGDFAELYVFKWTSLLIPPTTVLVINLVGMVAGISYAINSGYQSWGPLFGKLFFSIWVILHLYPFLKGLMGRQNRTPTIVIVWSILLASIFSLLWV

SEQ ID NO: 9 - protein, 249 aa, Oryza sativa
LNLYRIVIILRLIILMFFFQYRVTHPVRDAYGLWLVSVICEIWFALSWLLITSIPLIAYCVLPAICLLTNKFIIPEISNYAGMFFILLFASIFATGILELRWSGVGIEDWWRNEQFWVIGGTSAHLFAVFQGLLKVLAGIDTNFTVTSKASDEDGDFAELYVFKWTSLLIPPTTVLVINLVGMVAGISYAINSGYQSWGPLFGKLFFSIWVILHLYPFLKGLMGRQNRTPTIVIVWSILLASIFSLLWV

SEQ ID NO: 10 - protein, 85 aa, Arabidopsis thaliana
WTTLLIPPTTLLIVNLVGVVAGVSYAINSGYQSWGPLFGKLFFAFWVIVHLYPFLKGLMGRQNRTPTIVVVWSVLLASIFSLLWV

SEQ ID NO: 11 - protein, 85 aa, Glycine max
WTTLLIPPTTLLIINLVGVVAGISYAINSGYQSWGPLFGKLFFAFWVIIHLYPFLKGLMGRQNRTPTIVVVWSVLLASIFSLLWV

SEQ ID NO: 12 - protein, 85 aa, Fragaria vesca
WTTLLIPPTTLLIINLVGVVAGISYAVNSGYQSWGPLFGKLFFAFWVIVHLYPFLKGLMGRQNRTPTIVVVWSVLLASIFSLLWV

SEQ ID NO: 13 - protein, 85 aa, Vitis vinifera
WTTLLIPPTTLLIINLVGVVAGISYAINSGYQSWGPLFGKLFFAFWVIVHLYPFLKGLMGRQNRTPTIVVVWSILLASIFSLLWV

SEQ ID NO: 14 - protein, 85 aa, Solanum lycopersicum
WTTLLIPPTTLLIVNLVGVVAGISYAVNSGYQSWGPLFGKLFFAFWVIVHLYPFLKGLMGRQNRTPTIVVVWSILLASIFSLLWV

SEQ ID NO: 15 - protein, 85 aa, Zea mays
WTTLLIPPTTVLVINLVGIVAGVSYAINSGYQSWGPLFGKLFFAIWVILHLYPFLKGLMGKQNRTPTIVIVWSVLLASIFSLLWV

SEQ ID NO: 16 - protein, 85 aa, Oryza sativa
WTTLLIPPTTILIINLVGVVAGISYAINSGYQSWGPLFGKLFFAFWVIVHLYPFLKGLMGRQNRTPTIVVVWAILLASIFSLLWV